European Patent Specification EP 4 070 092 B1, published August 30, 2023. Title: METHOD. Applicant: OXFORD NANOPORE TECHNOLOGIES LIMITED. The sequence listing filed with the application follows.

SEQUENCE LISTING (24 sequences)

SEQ ID NO: 1 - protein, 485 aa, Escherichia coli
MMNDGKQQSTFLFHDYETFGTHPALDRPAQFAAIRTDSEFNVIGEPEVFYCKPADDYLPQPGAVLITGITPQEARAKGENEAAFAARIHSLFTVPKTCILGYNNVRFDDEVTRNIFYRNFYDPYAWSWQHDNSRWDLLDVMRACYALRPEGINWPENDDGLPSFRLEHLTKANGIEHSNAHDAMADVYATIAMAKLVKTRQPRLFDYLFTHRNKHKLMALIDVPQMKPLVHVSGMFGAWRGNTSWVAPLAWHPENRNAVIMVDLAGDISPLLELDSDTLRERLYTAKTDLGDNAAVPVKLVHINKCPVLAQANTLRPEDADRLGINRQHCLDNLKILRENPQVREKVVAIFAEAEPFTPSDNVDAQLYNGFFSDADRAAMKIVLETEPRNLPALDITFVDKRIEKLLFNYRARNFPGTLDYAEQQRWLEHRRQVFTPEFLQGYADELQMLVQQYADDKEKVALLKALWQYAEEIVSGSGHHHHHH

SEQ ID NO: 2 - protein, 268 aa, Escherichia coli
MKFVSFNINGLRARPHQLEAIVEKHQPDVIGLQETKVHDDMFPLEEVAKLGYNVFYHGQKGHYGVALLTKETPIAVRRGFPGDDEEAQRRIIMAEIPSLLGNVTVINGYFPQGESRDHPIKFPAKAQFYQNLQNYLETELKRDNPVLIMGDMNISPTDLDIGIGEENRKRWLRTGKCSFLPEEREWMDRLMSWGLVDTFRHANPQTADRFSWFDYRSKGFDDNRGLRIDLLLASQPLAECCVETGIDYEIRSMEKPSDHAPVWATFRR

SEQ ID NO: 3 - protein, 425 aa, Thermus thermophilus
MFRRKEDLDPPLALLPLKGLREAAALLEEALRQGKRIRVHGDYDADGLTGTAILVRGLAALGADVHPFIPHRLEEGYGVLMERVPEHLEASDLFLTVDCGITNHAELRELLENGVEVIVTDHHTPGKTPPPGLVVHPALTPDLKEKPTGAGVAFLLLWALHERLGLPPPLEYADLAAVGTIADVAPLWGWNRALVKEGLARIPASSWVGLRLLAEAVGYTGKAVEVAFRIAPRINAASRLGEAEKALRLLLTDDAAEAQALVGELHRLNARRQTLEEAMLRKLLPQADPEAKAIVLLDPEGHPGVMGIVASRILEATLRPVFLVAQGKGTVRSLAPISAVEALRSAEDLLLRYGGHKEAAGFAMDEALFPAFKARVEAYAARFPDPVREVALLDLLPEPGLLPQVFRELALLEPYGEGNPEPLFL

SEQ ID NO: 4 - protein, 226 aa, Bacteriophage lambda
MTPDIILQRTGIDVRAVEQGDDAWHKLRLGVITASEVHNVIAKPRSGKKWPDMKMSYFHTLLAEVCTGVAPEVNAKALAWGKQYENDARTLFEFTSGVNVTESPIIYRDESMRTACSPDGLCSDGNGLELKCPFTSRDFMKFRLGGFEAIKSAYMAQVQYSMWVTRKNAWYFANYDPRMKREGLHYVVIERDEKYMASFDEIVPEFIEKMDEALAEIGFVFGEQWR

SEQ ID NO: 5 - protein, 608 aa, Bacillus subtilis phage Phi 29
MKHMPRKMYSCAFETTTKVEDCRVWAYGYMNIEDHSEYKIGNSLDEFMAWVLKVQADLYFHNLKFDGAFIINWLERNGFKWSADGLPNTYNTIISRMGQWYMIDICLGYKGKRKIHTVIYDSLKKLPFPVKKIAKDFKLTVLKGDIDYHKERPVGYKITPEEYAYIKNDIQIIAEALLIQFKQGLDRMTAGSDSLKGFKDIITTKKFKKVFPTLSLGLDKEVRYAYRGGFTWLNDRFKEKEIGEGMVFDVNSLYPAQMYSRLLPYGEPIVFEGKYVWDEDYPLHIQHIRCEFELKEGYIPTIQIKRSRFYKGNEYLKSSGGEIADLWLSNVDLELMKEHYDLYNVEYISGLKFKATTGLFKDFIDKWTYIKTTSEGAIKQLAKLMLNSLYGKFASNPDVTGKVPYLKENGALGFRLGEEETKDPVYTPMGVFITAWARYTTITAAQACYDRIIYCDTDSIHLTGTEIPDVIKDIVDPKKLGYWAHESTFKRAKYLRQKTYIQDIYMKEVDGKLVEGSPDDYTDIKFSVKCAGMTDKIKKEVTFENFKVGFSRKMKPKPVQVPGGVVLVDDTFTIKSGGSAWSHPQFEKGGGSGGGSGGSAWSHPQFEK

SEQ ID NO: 6 - protein, 970 aa, Citromicrobium bathyomarinum
MLSVANVRSPSAAASYFASDNYYASADADRSGQWIGDGAKRLGLEGKVEARAFDALLRGELPDGSSVGNPGQAHRPGTDLTFSVPKSWSLLALVGKDERIIAAYREAVVEALHWAEKNAAETRVVEKGMVVTQATGNLAIGLFQHDTNRNQEPNLHFHAVIANVTQGKDGKWRTLKNDRLWQLNTTLNSIAMARFRVAVEKLGYEPGPVLKHGNFEARGISREQVMAFSTRRKEVLEARRGPGLDAGRIAALDTRASKEGIEDRATLSKQWSEAAQSIGLDLKPLVDRARTKALGQGMEATRIGSLVERGRAWLSRFAAHVRGDPADPLVPPSVLKQDRQTIAAAQAVASAVRHLSQREAAFERTALYKAALDFGLPTTIADVEKRTRALVRSGDLIAGKGEHKGWLASRDAVVTEQRILSEVAAGKGDSSPAITPQKAAASVQAAALTGQGFRLNEGQLAAARLILISKDRTIAVQGIAGAGKSSVLKPVAEVLRDEGHPVIGLAIQNTLVQMLERDTGIGSQTLARFLGGWNKLLDDPGNVALRAEAQASLKDHVLVLDEASMVSNEDKEKLVRLANLAGVHRLVLIGDRKQLGAVDAGKPFALLQRAGIARAEMATNLRARDPVVREAQAAAQAGDVRKALRHLKSHTVEARGDGAQVAAETWLALDKETRARTSIYASGRAIRSAVNAAVQQGLLASREIGPAKMKLEVLDRVNTTREELRHLPAYRAGRVLEVSRKQQALGLFIGEYRVIGQDRKGKLVEVEDKRGKRFRFDPARIRAGKGDDNLTLLEPRKLEIHEGDRIRWTRNDHRRGLFNADQARVVEIANGKVTFETSKGDLVELKKDDPMLKRIDLAYALNVHMAQGLTSDRGIAVMDSRERNLSNQKTFLVTVTRLRDHLTLVVDSADKLGAAVARNKGEKASAIEVTGSVKPTATKGSGVDQPKSVEANKAEKELTRSKSKTLDFGI

SEQ ID NO: 7 - protein, 760 aa, Methanococcoides burtonii
MMIRELDIPRDIIGFYEDSGIKELYPPQAEAIEMGLLEKKNLLAAIPTASGKTLLAELAMIKAIREGGKALYIVPLRALASEKFERFKELAPFGIKVGISTGDLDSRADWLGVNDIIVATSEKTDSLLRNGTSWMDEITTVVVDEIHLLDSKNRGPTLEVTITKLMRLNPDVQVVALSATVGNAREMADWLGAALVLSEWRPTDLHEGVLFGDAINFPGSQKKIDRLEKDDAVNLVLDTIKAEGQCLVFESSRRNCAGFAKTASSKVAKILDNDIMIKLAGIAEEVESTGETDTAIVLANCIRKGVAFHHAGLNSNHRKLVENGFRQNLIKVISSTPTLAAGLNLPARRVIIRSYRRFDSNFGMQPIPVLEYKQMAGRAGRPHLDPYGESVLLAKTYDEFAQLMENYVEADAEDIWSKLGTENALRTHVLSTIVNGFASTRQELFDFFGATFFAYQQDKWMLEEVINDCLEFLIDKAMVSETEDIEDASKLFLRGTRLGSLVSMLYIDPLSGSKIVDGFKDIGKSTGGNMGSLEDDKGDDITVTDMTLLHLVCSTPDMRQLYLRNTDYTIVNEYIVAHSDEFHEIPDKLKETDYEWFMGEVKTAMLLEEWVTEVSAEDITRHFNVGEGDIHALADTSEWLMHAAAKLAELLGVEYSSHAYSLEKRIRYGSGLDLMELVGIRGVGRVRARKLYNAGFVSVAKLKGADISVLSKLVGPKVAYNILSGIGVRVNDKHFNSAPISSNTLDTLLDKNQKTFNDFQ

SEQ ID NO: 8 - protein, 439 aa, Enterobacteria phage T4
MTFDDLTEGQKNAFNIVMKAIKEKKHHVTINGPAGTGKTTLTKFIIEALISTGETGIILAAPTHAAKKILSKLSGKEASTIHSILKINPVTYEENVLFEQKEVPDLAKCRVLICDEVSMYDRKLFKILLSTIPPWCTIIGIGDNKQIRPVDPGENTAYISPFFTHKDFYQCELTEVKRSNAPIIDVATDVRNGKWIYDKVVDGHGVRGFTGDTALRDFMVNYFSIVKSLDDLFENRVMAFTNKSVDKLNSIIRKKIFETDKDFIVGEIIVMQEPLFKTYKIDGKPVSEIIFNNGQLVRIIEAEYTSTFVKARGVPGEYLIRHWDLTVETYGDDEYYREKIKIISSDEELYKFNLFLGKTAETYKNWNKGGKAPWSDFWDAKSQFSKVKALPASTFHKAQGMSVDRAFIYTPCIHYADVELAQQLLYVGVTRGRYDVFYV

SEQ ID NO: 9-10 - skipped (2 entries)

SEQ ID NO: 11 - DNA, 60 bp, Artificial Sequence
  nucleotide sequence of first polynucleotide strand of Y adaptor discussed in example 1
  misc_feature (1)..(1): 30x C3 spacers at 5'
  misc_feature (33)..(34): iSp18 spacer
  misc_feature (60)..(60): 3' BCN
gcaatcgtcgaatgcgtacgtcgttttttttttaatgtacttcgttcagttacgtattgc

SEQ ID NO: 12 - DNA, 41 bp, Artificial Sequence
  nucleotide sequence of second polynucleotide strand of Y adaptor discussed in example 1
cgacgtacgcattcgacgattgctttgaggcgagcggtcaa

SEQ ID NO: 13 - DNA, 27 bp, Artificial Sequence
  nucleotide sequence of third polynucleotide strand of Y adaptor discussed in example 1
  misc_feature (23)..(23): iBNA-A
  misc_feature (24)..(24): iBNA-meC
  misc_feature (25)..(25): iBNA-A
  misc_feature (26)..(26): iBNA-T
  misc_feature (27)..(27): 3BNA-T
gcaatacgtaactgaacgaagtacatt

SEQ ID NO: 14 - DNA, 44 bp, Artificial Sequence
  first polynucleotide strand used in the production of a dsDNA tail as discussed in Example 1
  misc_feature (1)..(1): 5' BCN
aatgtacttcgttcagttacgtattgctgcttgggtgtttaacc

SEQ ID NO: 15 - DNA, 44 bp, Artificial Sequence; identical to SEQ ID NO: 14
  second polynucleotide strand used in the production of a dsDNA tail as discussed in Example 1
  misc_feature (1)..(1): 5' trans-cyclooctene

SEQ ID NO: 16 - DNA, 44 bp, Artificial Sequence
  polynucleotide strand used in the production of a dsDNA tail as discussed in Example 2
ggttaaacacccaagcagcaatacgtaactgaacgaagtacatt

SEQ ID NO: 17-19 - skipped (3 entries)

SEQ ID NO: 20 - protein, 10 aa, Artificial Sequence
  first peptide fragment used in the production of a first polynucleotide-polypeptide construct as discussed in Example 1
  MISC_FEATURE (1)..(1): N-terminal azidoacetyl
  MISC_FEATURE (10)..(10): C-terminal ethylene diamine - azidoacetyl
GGSGDDSGSG

SEQ ID NO: 21 - protein, 10 aa, Artificial Sequence
  second peptide fragment used in the production of a second polynucleotide-polypeptide construct as discussed in Example 1
  MISC_FEATURE (1)..(1): N-terminal azidoacetyl
  MISC_FEATURE (10)..(10): C-terminal ethylene diamine - azidoacetyl
GGSGRRSGSG

SEQ ID NO: 22 - protein, 10 aa, Artificial Sequence
  third peptide fragment used in the production of a third polynucleotide-polypeptide construct as discussed in Example 1
  MISC_FEATURE (1)..(1): N-terminal azidoacetyl
  MISC_FEATURE (10)..(10): C-terminal ethylene diamine - azidoacetyl
GGSGYYSGSG

SEQ ID NO: 23 - protein, 10 aa, Artificial Sequence
  peptide fragment used in the production of a polynucleotide-polypeptide construct as discussed in Example 2
GGSGDDSGSC

SEQ ID NO: 24 - protein, 21 aa, Artificial Sequence
  peptide fragment used in the production of a polynucleotide-polypeptide construct as discussed in Example 3
GDDDGSASGDDDGSASGDDDG